European Patent Application EP 4 342 995 A2, published March 27, 2024. Title: Methods for controlling blood pharmacokinetics of antibodies. Applicant: CHUGAI SEIYAKU KABUSHIKI KAISHA. The sequence listing filed with the application follows.

SEQUENCE LISTING (18 sequences)

SEQ ID NO: 1 - DNA, 354 bp, synthetic construct
  source 1..354: mol_type = other DNA; note = An artificially synthesized nucleotide sequence
caggtccagcttgtgcagtctggggctgaggtgaagaagcctgggtcctcagtgaaggtttcctgcaaggcctctggaggcaccttcagtgactactatatgcactgggtgcgccaggcccccggacaagggcttgagtggatgggatacattaatcctagcagtggttatactaagtacaatcggaagttcagggacagagtcaccattaccgcggacaaatccacgagcacagcctacatggagctgagcagcctgagatctgaagacacggctgtgtattactgtgcgagagggggtaacggttactaccttgactactggggccagggcaccacggtcaccgtctcctca

SEQ ID NO: 2 - protein, 118 aa, synthetic construct
  source 1..118: note = An artificially synthesized peptide sequence
QVQLVQSGAEVKKPGSSVKVSCKASGGTFSDYYMHWVRQAPGQGLEWMGYINPSSGYTKYNRKFRDRVTITADKSTSTAYMELSSLRSEDTAVYYCARGGNGYYLDYWGQGTTVTVSS

SEQ ID NO: 3 - DNA, 357 bp, synthetic construct
  source 1..357: mol_type = other DNA; note = An artificially synthesized nucleotide sequence
caggtgcagctggtgcagtctggacctgacgtgaagaagccgggggcctcagtgaaggtctcctgcaaggcctctggctacatgttttccgacaacaacatggactgggcgcgacaggcccctggacaagggcttgagtggatgggagatattaatactaaaagtggtggttctatctacaaccagaagttcaagggcagagtcatcatgaccatagacaaatccacgggcacagcctacatggaattgaggagcctgagatcagacgacacggccatatattactgtgcgaggaggaggagctacggctactactttgactactggggccagggaaccctggtcaccgtctcctca

SEQ ID NO: 4 - protein, 119 aa, synthetic construct
  source 1..119: note = An artificially synthesized peptide sequence
QVQLVQSGPDVKKPGASVKVSCKASGYMFSDNNMDWARQAPGQGLEWMGDINTKSGGSIYNQKFKGRVIMTIDKSTGTAYMELRSLRSDDTAIYYCARRRSYGYYFDYWGQGTLVTVSS

SEQ ID NO: 5 - DNA, 318 bp, synthetic construct
  source 1..318: mol_type = other DNA; note = An artificially synthesized nucleotide sequence
gacatcgtgatgacccagtctccatcctccctgtctgcatctgtaggagacagagtcaccatcacttgcaaggccagtcagaatgtggggactgctgtagcctggtatcagcagaaaccagggaaagcccctaagctcctgatctattcggcatcctaccggtacagtggggtcccatcaaggttcagtggcagtcgatatgggacagatttcactctcaccatctcaagcttgcaacctgaagatttagcaacttactactgtcagcaatatagcaactatatcacgttcggcggagggaccaaggtggagatcaaa

SEQ ID NO: 6 - protein, 106 aa, synthetic construct
  source 1..106: note = An artificially synthesized peptide sequence
DIVMTQSPSSLSASVGDRVTITCKASQNVGTAVAWYQQKPGKAPKLLIYSASYRYSGVPSRFSGSRYGTDFTLTISSLQPEDLATYYCQQYSNYITFGGGTKVEIK

SEQ ID NO: 7 - protein, 118 aa, synthetic construct
  source 1..118: note = An artificially synthesized peptide sequence
QVQLVQSGAEVKKPGSSVKVSCKASGGTFSDYYMHWVRQAPGEGLEWMGYINPSSGYTKYNRKFRDRVTITADKSTSTAYMELSSLRSEDTAVYYCARGGNGYYLDYWGEGTTVTVSS

SEQ ID NO: 8 - protein, 106 aa, synthetic construct
  source 1..106: note = An artificially synthesized peptide sequence
DIVMTQSPSSLSASVGDRVTITCKASQNVGTAVAWYQQKPGKAPKLLIYSASYRYSGVPSRFSGSRYGTDFTLTISSLQPEDLATYYCQQYSNYITFGQGTKVEIK

SEQ ID NO: 9 - protein, 118 aa, synthetic construct
  source 1..118: note = An artificially synthesized peptide sequence
QVQLVQSGAEVKKPGSSVKVSCKASGGTFSDYYMHWVRQAPGQGLEWMGYINPSSGYTKYNRKFRDRVTITADKSTSTAYMELSSLRSEDTAVYYCARGGRGYYLDYWGQGTTVTVSS

SEQ ID NO: 10 - protein, 119 aa, synthetic construct
  source 1..119: note = An artificially synthesized peptide sequence
QVQLVQSGPDVKKPGASVKVSCKASGYMFSDNNMDWARKAPGKGLEWMGDINTKSGGSIYNQKFKGRVIMTIDKSTGTAYMELRSLRSDDTAIYYCARRRSYGYYFDYWGRGTLVTVSS

SEQ ID NO: 11 - protein, 118 aa, synthetic construct
  source 1..118: note = An artificially synthesized peptide sequence
EVQLVQSGAEVVKPGSSVKVSCTASGYTFSDYYMHWVRQAPGEGLEWMGYINPSSGYTKYNRKFRDRVTITADKSTSTAYMELSSLRSEDTAVYYCARGGLGYYLDYWGEGTTVTVSS

SEQ ID NO: 12 - protein, 119 aa, synthetic construct
  source 1..119: note = An artificially synthesized peptide sequence
EVQLVQSGAQVKKPGASVKVSCKASGYTFSDNNMDWVRQAPGKGLEWMGDINTKSGGSIYNQKFKGRVIMTIDKSTGTAYMELRSLRSDDTAIYYCARRRSYGYYFDYWGRGTLVTVSS

SEQ ID NO: 13 - protein, 463 aa, Homo sapiens
MDWTWRFLFVVAAATGVQSQVQLLESGAVLARPGTSVKISCKASGFNIKDYYMHWVKQRPGQGLEWIGGNDPANGHSMYDPKFQGRVTITADTSTSTVFMELSSLRSEDTAVYYCARDSGYAMDYWGQGTLVTVSSASTKGPSVFPLAPCSRSTSESTAALGCLVKDYFPEPVTVSWNSGALTSGVHTFPAVLQSSGLYSLSSVVTVPSSSLGTKTYTCNVDHKPSNTKVDKRVESKYGPPCPPCPAPEFLGGPSVFLFPPKPKDTLMISRTPEVTCVVVDVSQEDPEVQFNWYVDGVEVHNAKTKPREEQFNSTYRVVSVLTVLHQDWLNGKEYKCKVSNKGLPSSIEKTISKAKGQPREPQVYTLPPSQEEMTKNQVSLTCLVKGFYPSDIAVEWESNGQPENNYKTTPPVLDSDGSFFLYSRLTVDKSRWQEGNVFSCSVMHEALHNHYTQKSLSLSLGK

SEQ ID NO: 14 - protein, 236 aa, Homo sapiens
MDMRVPAQLLGLLLLWLRGARCDIQMTQSPSSLSASVGDRVTITCKASQDIKSFLSWYQQKPEKAPKSLIYYATSLADGVPSRFSGSGSGTDYTLTISSLQPEDFATYYCLQHGESPYTFGGGTKVEIKRTVAAPSVFIFPPSDEQLKSGTASVVCLLNNFYPREAKVQWKVDNALQSGNSQESVTEQDSKDSTYSLSSTLTLSKADYEKHKVYACEVTHQGLSSPVTKSFNRGEC

SEQ ID NO: 15 - protein, 119 aa, Mus musculus
MEVQLQQSGAELVKPGASVKLSCTASGFNIKDYYMHWIKQRPGQGLEWLGYINPSSGYTKYNRKFRDKATLTADKSSSTAYMQLTSLTYEDSAVYYCARGGNGYYLDYWGQGTTLTVSS

SEQ ID NO: 16 - protein, 120 aa, Mus musculus
MQVQLQQSGPELVKPGASVKISCKASGYTFTDNNMDWVKQSHGKGLEWIGDINTKSGGSIYNQKFKGKATLTIDKSSSTAYMELRSLTSEDTAVYYCARRRSYGYYFDYWGQGTTLTVSS

SEQ ID NO: 17 - protein, 107 aa, Homo sapiens
DIVMTQSHKFMSTSVGDRVSITCKASQNVGTAVAWYQQKPGQSPKLLIYSASYRYSGVPDRFTGSRYGTDFTLTISNVQSEDLADYLCQQYSNYITFGGGTKLELKR

SEQ ID NO: 18 - protein, 108 aa, Mus musculus
DIVLTQSQKFMSTSVGDRVSITCKASQNVGTAVAWYQQKPGQSPKALIYSASYRYSGVPDRFTGSGSGTDFTLTISNVQSEDLAEYFCQQYNSYPLTFGAGTKLEIKR